European Patent Specification EP 3 064 506 B1, published October 18, 2023. Title: Method of Inhibitiion of Photo-crosslinking, and Self-crosslinking Inhibitory Type Photo-responsive Nucleic Acid. Applicant: Japan Advanced Institute of Science and Technology. The sequence listing filed with the application follows.

SEQUENCE LISTING (3 sequences)

SEQ ID NO: 1 - DNA, 12 bp, Artificial Sequence
  ODN 4
  Inventor: FUJIMOTO, Kenzo Inventor: NAKAMURA, Shigetaka
  misc_feature (4)..(4): n is cnvK
gtanagagtgta

SEQ ID NO: 2 - DNA, 12 bp, Artificial Sequence
  ODN 5
  misc_feature (2)..(2): n is cnT
  misc_feature (4)..(4): n is cnvK
  misc_feature (9)..(9): n is cnT
  misc_feature (11)..(11): n is cnT
gnanagagngna

SEQ ID NO: 3 - DNA, 20 bp, Artificial Sequence
  ODN 6
agagtacactctatactgag